European Patent Application EP 4 393 521 A1, published July 3, 2024. Title: BIONIC CORNEA AND PREPARATION METHOD THEREFOR. Applicant: EOSVISION MEDTECH TECHNOLOGY CO., LTD. The sequence listing filed with the application follows.

SEQUENCE LISTING (3 sequences)

SEQ ID NO: 1 - protein, 36 aa, Artificial Sequence
  misc_feature (14)..(14): Xaa can be any naturally occurring amino acid
  misc_feature (17)..(17): Xaa can be any naturally occurring amino acid
  misc_feature (20)..(20): Xaa can be any naturally occurring amino acid
  misc_feature (23)..(23): Xaa can be any naturally occurring amino acid
  misc_feature (26)..(26): Xaa can be any naturally occurring amino acid
  misc_feature (29)..(29): Xaa can be any naturally occurring amino acid
  misc_feature (32)..(32): Xaa can be any naturally occurring amino acid
  misc_feature (35)..(35): Xaa can be any naturally occurring amino acid
PKGPKGPKGPKGPXGPXGPXGPXGDXGDXGDXGDXG

SEQ ID NO: 2 - protein, 2 aa, Artificial Sequence
GC

SEQ ID NO: 3 - protein, 2 aa, Artificial Sequence
GF